European Patent Application EP 4 810 507 A1, published September 23, 2026. Title: Process for the removal of a monomethoxytrityl protecting group from a monomethoxytrityl protected amino linker moiety attached to an oligonucleotide. Applicant: F: Hoffmann-La Roche AG. Application EP. The sequence listing filed with the application follows.

SEQUENCE LISTING (1 sequence)

SEQ ID NO: 1 - DNA, 21 bp, synthetic construct
  source 1..21: mol_type = other DNA
atcccacgccccctgtccagc